European Patent Application EP 4 588 937 A1, published July 23, 2025. Title: USE OF NKG2D-BASED CELL ADAPTER MOLECULE IN REMOVAL OF AGING CELLS. Applicant: WEST CHINA HOSPITAL, SICHUAN UNIVERSITY. The sequence listing filed with the application follows.

SEQUENCE LISTING (5 sequences)

SEQ ID NO: 1 - protein, 139 aa, Homo sapiens
FLNSLFNQEVQIPLTESYCGPCPKNWICYKNNCYQFFDESKNWYESQASCMSQNASLLKVYSKEDQDLLKLVKSYHWMGLVHIPTNGSWQWEDGSILSPNLLTIIEMQKGDCALYASSFKGYIENCSTPNTYICMQRTV

SEQ ID NO: 2 - protein, 243 aa, synthetic construct
  source 1..243: note = CD3-binding domain
DIKLQQSGAELARPGASVKMSCKTSGYTFTRYTMHWVKQRPGQGLEWIGYINPSRGYTNYNQKFKDKATLTTDKSSSTAYMQLSSLTSEDSAVYYCARYYDDHYCLDYWGQGTTLTVSSVEGGSGGSGGSGGSGGVDDIQLTQSPAIMSASPGEKVTMTCRASSSVSYMNWYQQKSGTSPKRWIYDTSKVASGVPYRFSGSGSGTSYSLTISSMEAEDAATYYCQQWSSNPLTFGAGTKLELK

SEQ ID NO: 3 - protein, 241 aa, synthetic construct
  source 1..241: note = CD16-binding scFv
QVQLVQSGAEVKKPGESLKVSCKASGYTFTSYYMHWVRQAPGQGLEWMGIINPSGGSTSYAQKFQGRVTMTRDTSTSTVYMELSSLRSEDTAVYYCARGSAYYYDFADYWGQGTLVTVSSGGGGSGGGGSGGGGSSYVLTQPSSVSVAPGQTATISCGGHNIGSKNVHWYQQRPGQSPVLVIYQDNKRPSGIPERFSGSNSGNTATLTISGTQAMDEADYYCQVWDNYSVLFGGGTKLTVL

SEQ ID NO: 4 - protein, 120 aa, synthetic construct
  source 1..120: note = CD16-binding VhH
EVQLVESGGGFVQAGESLTLSCTSSTLTFTPYRMAWYRQAPGKQRDLVADISSGDGRTTNYADFAKGRFTISRDNIKNTVFLRMTNLKPEDTAVYYCNTFVSFVGIARSWGQGTQVTVSS

SEQ ID NO: 5 - protein, 231 aa, synthetic construct
  source 1..231: note = IgG Fc
PKSCDKTHTCPPCPAPELVGGPSVFLLPPKPKDTLMISRTPEVTCVVVDVSHEDPEVKFNWYVDGVEVHNAKTKPPEEQYNSTLRVVSVLTVLHQDWLNGKEYKCKVSNKALPAPIEKTISKAKGQPREPQVYTLPPSRDELTKNQVSLTCLVKGFYPSDIAVEWESNGQPENNYKTTPLVLDSDGSFFLYSKLTVDKSRWQQGNVFSCSVMHEALHNHYTQKSLSLSPGK